European Patent Application EP 4 726 384 A1, published April 15, 2026. Title: Methods for detecting soy. Applicant: NISSIN FOODS HOLDINGS. Application JP PNSH-00795. The sequence listing filed with the application follows.

SEQUENCE LISTING (3 sequences)

SEQ ID NO: 1 - protein, 12 aa, Glycine max
SQSDNFEYVSFK

SEQ ID NO: 2 - protein, 13 aa, Glycine max
VLIVPQNFVVAAR

SEQ ID NO: 3 - protein, 13 aa, Glycine max
FYLAGNQEQEFLK